European Patent Application EP 4 588 483 A2, published July 23, 2025. Title: COVALENT ADAPTOR SYNNOTCH AND CHIMERIC ANTIGEN RECEPTORS (CARS) FOR PROGRAMMABLE ANTIGEN-TARGETING. Applicant: University of Pittsburgh - of the Commonwealth System of Higher Education. The sequence listing filed with the application follows.

SEQUENCE LISTING (9 sequences)

SEQ ID NO: 1 - DNA, 2067 bp, synthetic construct
  misc_feature 1..2067: note = Synthetic construct
  source 1..2067: mol_type = other DNA
atggagacagacacactcctgctatgggtgctgctgctctgggttccaggttccacaggtatggacaaagattgcgagatgaagagaaccaccctggatagccctctcggcaagctcgaactttctggttgtgaacagggtttgcacaggatcatcttcctgggaaagggaacctcagccgcagatgcggttgaagtgccagctccggctgcagtgcttggtggacccgagcctcttatgcaagcaacggcatggcttaatgcttattttcaccagcctgaggccattgaagagtttccagttcctgcattgcatcaccccgtttttcagcaggaatccttcactagacaagtgctttggaagctcttgaaagtggttaaatttggggaagtcatctcatacagccaccttgctgcccttgcaggcaatcctgcggccacggctgcagtgaaaactgcacttagcggaaatccagtccccatcttgataccgtgtcacagggtagtacagggcgacctggacgtcggcggttacgagggcggtttggccgttaaggaatggttgctggcgcatgagggtcaccggctgggaaaaccaggtcttggtggaggaagtggaggatctaccactactccggcaccgcgccccccaactcctgcaccgacgatagcttcacaaccgctttcattgcggcccgaagcatgtcggccagccgccggaggcgctgtgcatacaagagggctggattttgcatgtgatatatatatttgggcgccccttgctggcacttgcggcgttcttcttcttagcctcgttattacgctctactgtaagcgaggtaggaaaaaattgctgtatatctttaaacagccttttatgagacccgtgcaaacgactcaagaggaagacgggtgtagctgtagatttcctgaagaggaagagggggggtgcgaactgcgggtgaagttcagcagaagcgccgacgcccctgcctaccagcagggccagaatcagctgtacaacgagctgaacctgggcagaagggaagagtacgacgtcctggataagcggagaggccgggaccctgagatgggcggcaagcctcggcggaagaacccccaggaaggcctgtataacgaactgcagaaagacaagatggccgaggcctacagcgagatcggcatgaagggcgagcggaggcggggcaagggccacgacggcctgtatcagggcctgtccaccgccaccaaggatacctacgacgccctgcacatgcaggccctgcccccaaggctcgagggcggcggagagggcagaggaagtcttctaacatgcggtgacgtggaggagaatcccggccctcgcatgagcgagctgattaaggagaacatgcacatgaagctgtacatggagggcaccgtggacaaccatcacttcaagtgcacatccgagggcgaaggcaagccctacgagggcacccagaccatgagaatcaaggtggtcgagggcggccctctccccttcgccttcgacatcctggctactagcttcctctacggcagcaagaccttcatcaaccacacccagggcatccccgacttcttcaagcagtccttccctgagggcttcacatgggagagagtcaccacatacgaagacgggggcgtgctgaccgctacccaggacaccagcctccaggacggctgcctcatctacaacgtcaagatcagaggggtgaacttcacatccaacggccctgtgatgcagaagaaaacactcggctgggaggccttcaccgagacgctgtaccccgctgacggcggcctggaaggcagaaacgacatggccctgaagctcgtgggcgggagccatctgatcgcaaacatcaagaccacatatagatccaagaaacccgctaagaacctcaagatgcctggcgtctactatgtggactacagactggaaagaatcaaggaggccaacaacgaaacatacgtcgagcagcacgaggtggcagtggccagatactgcgacctccctagcaaactggggcacaagcttaattaa

SEQ ID NO: 2 - DNA, 2271 bp, synthetic construct
  misc_feature 1..2271: note = Synthetic construct
  source 1..2271: mol_type = other DNA
atggcgctccctgtcaccgcactgcttcttccgctggcactgctgctgcacgctgcacggcctgagcaaaaacttatctctgaagaggacctcatggacaaagattgcgagatgaagagaaccaccctggatagccctctcggcaagctcgaactttctggttgtgaacagggtttgcacaggatcatcttcctgggaaagggaacctcagccgcagatgcggttgaagtgccagctccggctgcagtgcttggtggacccgagcctcttatgcaagcaacggcatggcttaatgcttattttcaccagcctgaggccattgaagagtttccagttcctgcattgcatcaccccgtttttcagcaggaatccttcactagacaagtgctttggaagctcttgaaagtggttaaatttggggaagtcatctcatacagccaccttgctgcccttgcaggcaatcctgcggccacggctgcagtgaaaactgcacttagcggaaatccagtccccatcttgataccgtgtcacagggtagtacagggcgacctggacgtcggcggttacgagggcggtttggccgttaaggaatggttgctggcgcatgagggtcaccggctgggaaaaccaggtcttggtggaggaagtggaggatctatcctggactacagcttcacaggtggcgctgggcgcgacattcccccaccgcagattgaggaggcctgtgagctgcctgagtgccaggtggatgcaggcaataaggtctgcaacctgcagtgtaataatcacgcatgtggctgggatggtggcgactgctccctcaacttcaatgacccctggaagaactgcacgcagtctctacagtgctggaagtattttagcgacggccactgtgacagccagtgcaactcggccggctgcctctttgatggcttcgactgccagctcaccgagggacagtgcaaccccctgtatgaccagtactgcaaggaccacttcagtgatggccactgcgaccagggctgtaacagtgccgaatgtgagtgggatggcctagactgtgctgagcatgtacccgagcggctggcagccggcaccctggtgctggtggtgctgcttccacccgaccagctacggaacaactccttccactttctgcgggagctcagccacgtgctgcacaccaacgtggtcttcaagcgtgatgcgcaaggccagcagatgatcttcccgtactatggccacgaggaagagctgcgcaagcacccaatcaagcgctctacagtgggttgggccacctcttcactgcttcctggtaccagtggtgggcgccagcgcagggagctggaccccatggacatccgtggctccattgtctacctggagatcgacaaccggcaatgtgtgcagtcatcctcgcagtgcttccagagtgccaccgatgtggctgccttcctaggtgctcttgcgtcacttggcagcctcaatattccttacaagattgaggccgtgaagagtgagccggtggagcctccgctgccctcgcagctgcacctcatgtacgtggcagcggccgccttcgtgctcctgttctttgtgggctgtggggtgctgctgtcccgcaagcgccggcggatgaagctgctgagcagcatcgagcaggcctgtgacatctgccggctgaagaaactgaagtgcagcaaagaaaagcccaagtgcgccaagtgcctgaagaacaactgggagtgccggtacagccccaagaccaagagaagccccctgaccagagcccacctgaccgaggtggaaagccggctggaaagactggaacagctgtttctgctgatcttcccacgcgaggacctggacatgatcctgaagatggacagcctgcaggacatcaaggccctgctgaccggcctgttcgtgcaggacaacgtgaacaaggacgccgtgaccgacagactggccagcgtggaaaccgacatgcccctgaccctgcggcagcacagaatcagcgccaccagcagcagcgaggaaagcagcaacaagggccagcggcagctgacagtgtctgctgctgcaggcggaagcggaggctctggcggatctgatgccctggacgacttcgacctggatatgctgggcagcgacgccctggatgattttgatctggacatgctgggatctgacgctctggacgatttcgatctcgacatgttgggatcagatgcactggatgactttgacctggacatgctcggatcatga

SEQ ID NO: 3 - DNA, 564 bp, synthetic construct
  misc_feature 1..564: note = Synthetic construct
  source 1..564: mol_type = other DNA
atggacaaagattgcgagatgaagagaaccaccctggatagccctctcggcaagctcgaactttctggttgtgaacagggtttgcacaggatcatcttcctgggaaagggaacctcagccgcagatgcggttgaagtgccagctccggctgcagtgcttggtggacccgagcctcttatgcaagcaacggcatggcttaatgcttattttcaccagcctgaggccattgaagagtttccagttcctgcattgcatcaccccgtttttcagcaggaatccttcactagacaagtgctttggaagctcttgaaagtggttaaatttggggaagtcatctcatacagccaccttgctgcccttgcaggcaatcctgcggccacggctgcagtgaaaactgcacttagcggaaatccagtccccatcttgataccgtgtcacagggtagtacagggcgacctggacgtcggcggttacgagggcggtttggccgttaaggaatggttgctggcgcatgagggtcaccggctgggaaaaccaggtcttggtggaggaagtggaggatct

SEQ ID NO: 4 - DNA, 336 bp, synthetic construct
  misc_feature 1..336: note = Synthetic construct
  source 1..336: mol_type = other DNA
cgggtgaagttcagcagaagcgccgacgcccctgcctaccagcagggccagaatcagctgtacaacgagctgaacctgggcagaagggaagagtacgacgtcctggataagcggagaggccgggaccctgagatgggcggcaagcctcggcggaagaacccccaggaaggcctgtataacgaactgcagaaagacaagatggccgaggcctacagcgagatcggcatgaagggcgagcggaggcggggcaagggccacgacggcctgtatcagggcctgtccaccgccaccaaggatacctacgacgccctgcacatgcaggccctgcccccaagg

SEQ ID NO: 5 - DNA, 978 bp, synthetic construct
  misc_feature 1..978: note = Synthetic construct
  source 1..978: mol_type = other DNA
atcctggactacagcttcacaggtggcgctgggcgcgacattcccccaccgcagattgaggaggcctgtgagctgcctgagtgccaggtggatgcaggcaataaggtctgcaacctgcagtgtaataatcacgcatgtggctgggatggtggcgactgctccctcaacttcaatgacccctggaagaactgcacgcagtctctacagtgctggaagtattttagcgacggccactgtgacagccagtgcaactcggccggctgcctctttgatggcttcgactgccagctcaccgagggacagtgcaaccccctgtatgaccagtactgcaaggaccacttcagtgatggccactgcgaccagggctgtaacagtgccgaatgtgagtgggatggcctagactgtgctgagcatgtacccgagcggctggcagccggcaccctggtgctggtggtgctgcttccacccgaccagctacggaacaactccttccactttctgcgggagctcagccacgtgctgcacaccaacgtggtcttcaagcgtgatgcgcaaggccagcagatgatcttcccgtactatggccacgaggaagagctgcgcaagcacccaatcaagcgctctacagtgggttgggccacctcttcactgcttcctggtaccagtggtgggcgccagcgcagggagctggaccccatggacatccgtggctccattgtctacctggagatcgacaaccggcaatgtgtgcagtcatcctcgcagtgcttccagagtgccaccgatgtggctgccttcctaggtgctcttgcgtcacttggcagcctcaatattccttacaagattgaggccgtgaagagtgagccggtggagcctccgctgccctcgcagctgcacctcatgtacgtggcagcggccgccttcgtgctcctgttctttgtgggctgtggggtgctgctgtcccgcaagcgccggcgg

SEQ ID NO: 6 - DNA, 2122 bp, synthetic construct
  misc_feature 1..2122: note = Synthetic construct
  source 1..2122: mol_type = other DNA
ggagcaaggcaggtggacagtggatcatggagacagacacactcctgctatgggtgctgctgctctgggttccaggttccacaggtatggacaaagattgcgagatgaagagaaccaccctggatagccctctcggcaagctcgaactttctggttgtgaacagggtttgcacaggatcatcttcctgggaaagggaacctcagccgcagatgcggttgaagtgccagctccggctgcagtgcttggtggacccgagcctcttatgcaagcaacggcatggcttaatgcttattttcaccagcctgaggccattgaagagtttccagttcctgcattgcatcaccccgtttttcagcaggaatccttcactagacaagtgctttggaagctcttgaaagtggttaaatttggggaagtcatctcatacagccaccttgctgcccttgcaggcaatcctgcggccacggctgcagtgaaaactgcacttagcggaaatccagtccccatcttgataccgtgtcacagggtagtacagggcgacctggacgtcggcggttacgagggcggtttggccgttaaggaatggttgctggcgcatgagggtcaccggctgggaaaaccaggtcttggtggaggaagtggaggatctaccactactccggcaccgcgccccccaactcctgcaccgacgatagcttcacaaccgctttcattgcggcccgaagcatgtcggccagccgccggaggcgctgtgcatacaagagggctggattttgcatgtgatatatatatttgggcgccccttgctggcacttgcggcgttcttcttcttagcctcgttattacgctctactgtaagcgaggtaggaaaaaattgctgtatatctttaaacagccttttatgagacccgtgcaaacgactcaagaggaagacgggtgtagctgtagatttcctgaagaggaagagggggggtgcgaactgcgggtgaagttcagcagaagcgccgacgcccctgcctaccagcagggccagaatcagctgtacaacgagctgaacctgggcagaagggaagagtacgacgtcctggataagcggagaggccgggaccctgagatgggcggcaagcctcggcggaagaacccccaggaaggcctgtataacgaactgcagaaagacaagatggccgaggcctacagcgagatcggcatgaagggcgagcggaggcggggcaagggccacgacggcctgtatcagggcctgtccaccgccaccaaggatacctacgacgccctgcacatgcaggccctgcccccaaggctcgagggcggcggagagggcagaggaagtcttctaacatgcggtgacgtggaggagaatcccggccctcgcatgagcgagctgattaaggagaacatgcacatgaagctgtacatggagggcaccgtggacaaccatcacttcaagtgcacatccgagggcgaaggcaagccctacgagggcacccagaccatgagaatcaaggtggtcgagggcggccctctccccttcgccttcgacatcctggctactagcttcctctacggcagcaagaccttcatcaaccacacccagggcatccccgacttcttcaagcagtccttccctgagggcttcacatgggagagagtcaccacatacgaagacgggggcgtgctgaccgctacccaggacaccagcctccaggacggctgcctcatctacaacgtcaagatcagaggggtgaacttcacatccaacggccctgtgatgcagaagaaaacactcggctgggaggccttcaccgagacgctgtaccccgctgacggcggcctggaaggcagaaacgacatggccctgaagctcgtgggcgggagccatctgatcgcaaacatcaagaccacatatagatccaagaaacccgctaagaacctcaagatgcctggcgtctactatgtggactacagactggaaagaatcaaggaggccaacaacgaaacatacgtcgagcagcacgaggtggcagtggccagatactgcgacctccctagcaaactggggcacaagcttaattaagatccttgacttgcggccgcaactcccac

SEQ ID NO: 7 - DNA, 624 bp, synthetic construct
  misc_feature 1..624: note = Synthetic construct
  source 1..624: mol_type = other DNA
gagcaaaaacttatctctgaagaggacctcatggacaaagattgcgagatgaagagaaccaccctggatagccctctcggcaagctcgaactttctggttgtgaacagggtttgcacaggatcatcttcctgggaaagggaacctcagccgcagatgcggttgaagtgccagctccggctgcagtgcttggtggacccgagcctcttatgcaagcaacggcatggcttaatgcttattttcaccagcctgaggccattgaagagtttccagttcctgcattgcatcaccccgtttttcagcaggaatccttcactagacaagtgctttggaagctcttgaaagtggttaaatttggggaagtcatctcatacagccaccttgctgcccttgcaggcaatcctgcggccacggctgcagtgaaaactgcacttagcggaaatccagtccccatcttgataccgtgtcacagggtagtacagggcgacctggacgtcggcggttacgagggcggtttggccgttaaggaatggttgctggcgcatgagggtcaccggctgggaaaaccaggtcttggtggaggaagtggaggatctatcctggactacagcttcacaggtggcgct

SEQ ID NO: 8 - DNA, 624 bp, synthetic construct; identical to SEQ ID NO: 7
  misc_feature 1..624: note = Synthetic construct
  source 1..624: mol_type = other DNA

SEQ ID NO: 9 - DNA, 591 bp, synthetic construct
  misc_feature 1..591: note = Synthetic construct
  source 1..591: mol_type = other DNA
ccgatccagcctctcgacattcgttggatcatgttccacgtaagtttcagatatatctttggacttccgccgctcatattggtattgttgccagtggcatctagtgactgtgacatagaaggaaaggatggtaaacagtatgaaagcgtacttatggtatccattgaccagcttctcgatagtatgaaagagattggtagtaattgcctcaataacgagttcaatttctttaaacgacacatttgtgatgcgaataaagagggaatgtttctgtttcgcgccgcgaggaagcttaggcagttccttaaaatgaactcaactggggatttcgacctccatctgctgaaggtgagtgaaggtactactattctcctgaattgcacgggacaggtaaaggggcgaaaacctgcggccttgggtgaggcacaaccaaccaaaagcctcgaagaaaacaagtccctcaaagaacagaagaagctcaacgatctgtgctttctgaaaagactcttgcaggagatcaaaacttgttggaataagattttgatgggcactaaggagcattaagatccttgacttgcggccgcaactccc